European Patent Specification EP 3 442 600 B1, published March 13, 2024. Title: ADENO-ASSOCIATED VIRUS VECTOR DELIVERY OF B-SARCOGLYCAN AND MICRORNA-29 AND THE TREATMENT OF MUSCULAR DYSTROPHY. Applicant: Research Institute at Nationwide Children's Hospital. The sequence listing filed with the application follows.

SEQUENCE LISTING (18 sequences)

SEQ ID NO: 1 - DNA, 957 bp, Homo sapiens
  misc_feature: Beta-sarcoglycan
atggcagcagcagccgccgcagccgccgagcagcagtcaagcaatggaccagtgaaaaaatcaatgagagaaaaagccgtcgagaggagatcagtgaataaggagcacaacagcaatttcaaagccggctacatccctattgacgaagatcgcctgcataagacaggcctgagggggcgcaaaggaaacctggcaatctgcgtcatcattctgctgtttatcctggccgtgattaatctgatcattactctggtgatttgggctgtcatccgcattggcccaaacgggtgtgactctatggagttccacgaaagtggcctgctgcgatttaagcaggtgtccgatatgggggtcatccatccactgtacaaatctactgtcggcgggcggagaaacgagaatctggtgatcaccgggaacaatcagcccattgtgttccagcagggaaccacaaagctgtctgtggaaaacaataaaacatcaatcactagcgacattggcatgcagttctttgatccccggacccagaatatcctgttcagtaccgactatgagacacacgaatttcatctgccttccggggtgaagtctctgaacgtccagaaagccagcactgagagaatcaccagtaacgctacatcagacctgaatatcaaggtggatggacgagctattgtccggggaaatgagggcgtgttcatcatgggcaagacaattgaatttcacatgggaggcaacatggagctgaaagcagaaaacagcatcattctgaatgggagcgtgatggtctccactaccagactgcccagctcctctagtggagaccagctggggtccggagattgggtcaggtataagctgtgcatgtgtgccgatggcaccctgtttaaagtgcaggtcaccagccagaatatgggatgtcagattagcgataacccttgtgggaatactcattaa

SEQ ID NO: 2 - protein, 318 aa, Homo sapiens
  MISC_FEATURE: Beta-sarcoglycan
MAAAAAAAAEQQSSNGPVKKSMREKAVERRSVNKEHNSNFKAGYIPIDEDRLHKTGLRGRKGNLAICVIILLFILAVINLIITLVIWAVIRIGPNGCDSMEFHESGLLRFKQVSDMGVIHPLYKSTVGGRRNENLVITGNNQPIVFQQGTTKLSVENNKTSITSDIGMQFFDPRTQNILFSTDYETHEFHLPSGVKSLNVQKASTERITSNATSDLNIKVDGRAIVRGNEGVFIMGKTIEFHMGGNMELKAENSIILNGSVMVSTTRLPSSSSGDQLGSGDWVRYKLCMCADGTLFKVQVTSQNMGCQISDNPCGNTH

SEQ ID NO: 3 - DNA, 2306 bp, Artificial Sequence
  Primer
  misc_feature: pAAV.MHCK7.hSCGB
ctgcgcgctcgctcgctcactgaggccgcccgggcaaagcccgggcgtcgggcgacctttggtcgcccggcctcagtgagcgagcgagcgcgcagagagggagtggggttaaccaattggcgcggccgcaagcttgcatgtctaagctagacccttcagattaaaaataactgaggtaagggcctgggtaggggaggtggtgtgagacgctcctgtctctcctctatctgcccatcggccctttggggaggaggaatgtgcccaaggactaaaaaaaggccatggagccagaggggcgagggcaacagacctttcatgggcaaaccttggggccctgctgtctagcatgccccactacgggtctaggctgcccatgtaaggaggcaaggcctggggacacccgagatgcctggttataattaacccagacatgtggctgcccccccccccccaacacctgctgcctctaaaaataaccctgtccctggtggatcccctgcatgcgaagatcttcgaacaaggctgtgggggactgagggcaggctgtaacaggcttgggggccagggcttatacgtgcctgggactcccaaagtattactgttccatgttcccggcgaagggccagctgtcccccgccagctagactcagcacttagtttaggaaccagtgagcaagtcagcccttggggcagcccatacaaggccatggggctgggcaagctgcacgcctgggtccggggtgggcacggtgcccgggcaacgagctgaaagctcatctgctctcaggggcccctccctggggacagcccctcctggctagtcacaccctgtaggctcctctatataacccaggggcacaggggctgccctcattctaccaccacctccacagcacagacagacactcaggagcagccagcggcgcgcccaggtaagtttagtctttttgtcttttatttcaggtcccggatccggtggtggtgcaaatcaaagaactgctcctcagtggatgttgcctttacttctaggcctgtacggaagtgttacttctgctctaaaagctgcggaattgtacccggtaccgccaccatggcagcagcagccgccgcagccgccgagcagcagtcaagcaatggaccagtgaaaaaatcaatgagagaaaaagccgtcgagaggagatcagtgaataaggagcacaacagcaatttcaaagccggctacatccctattgacgaagatcgcctgcataagacaggcctgagggggcgcaaaggaaacctggcaatctgcgtcatcattctgctgtttatcctggccgtgattaatctgatcattactctggtgatttgggctgtcatccgcattggcccaaacgggtgtgactctatggagttccacgaaagtggcctgctgcgatttaagcaggtgtccgatatgggggtcatccatccactgtacaaatctactgtcggcgggcggagaaacgagaatctggtgatcaccgggaacaatcagcccattgtgttccagcagggaaccacaaagctgtctgtggaaaacaataaaacatcaatcactagcgacattggcatgcagttctttgatccccggacccagaatatcctgttcagtaccgactatgagacacacgaatttcatctgccttccggggtgaagtctctgaacgtccagaaagccagcactgagagaatcaccagtaacgctacatcagacctgaatatcaaggtggatggacgagctattgtccggggaaatgagggcgtgttcatcatgggcaagacaattgaatttcacatgggaggcaacatggagctgaaagcagaaaacagcatcattctgaatgggagcgtgatggtctccactaccagactgcccagctcctctagtggagaccagctggggtccggagattgggtcaggtataagctgtgcatgtgtgccgatggcaccctgtttaaagtgcaggtcaccagccagaatatgggatgtcagattagcgataacccttgtgggaatactcattaaaagcttggccgcaataaaagatctttattttcattagatctgtgtgttggttttttgtgtgtcctgcaggggcgcgcctctagagcatggctacgtagataagtagcatggcgggttaatcattaactacaaggaacccctagtgatggagttggccactccctctctgcgcgctcgctcgctcactgaggccgggcgaccaaaggtcgcccgacgcccgggctttgcccgggcggcctcagtgagcgagcgagcgcgc

SEQ ID NO: 4 - DNA, 792 bp, Artificial Sequence
  Primer
  misc_feature: MHCK7 promoter
aagcttgcatgtctaagctagacccttcagattaaaaataactgaggtaagggcctgggtaggggaggtggtgtgagacgctcctgtctctcctctatctgcccatcggccctttggggaggaggaatgtgcccaaggactaaaaaaaggccatggagccagaggggcgagggcaacagacctttcatgggcaaaccttggggccctgctgtctagcatgccccactacgggtctaggctgcccatgtaaggaggcaaggcctggggacacccgagatgcctggttataattaacccagacatgtggctgcccccccccccccaacacctgctgcctctaaaaataaccctgtccctggtggatcccctgcatgcgaagatcttcgaacaaggctgtgggggactgagggcaggctgtaacaggcttgggggccagggcttatacgtgcctgggactcccaaagtattactgttccatgttcccggcgaagggccagctgtcccccgccagctagactcagcacttagtttaggaaccagtgagcaagtcagcccttggggcagcccatacaaggccatggggctgggcaagctgcacgcctgggtccggggtgggcacggtgcccgggcaacgagctgaaagctcatctgctctcaggggcccctccctggggacagcccctcctggctagtcacaccctgtaggctcctctatataacccaggggcacaggggctgccctcattctaccaccacctccacagcacagacagacactcaggagcagccagc

SEQ ID NO: 5 - DNA, 2244 bp, Artificial Sequence
  Primer
  misc_feature: pAAV.tMCK.hSGCB
ctgcgcgctcgctcgctcactgaggccgcccgggcaaagcccgggcgtcgggcgacctttggtcgcccggcctcagtgagcgagcgagcgcgcagagagggagtggggttaaccaattggcggccgcaaacttgcatgccccactacgggtctaggctgcccatgtaaggaggcaaggcctggggacacccgagatgcctggttataattaaccccaacacctgctgcccccccccccccaacacctgctgcctgagcctgagcggttaccccaccccggtgcctgggtcttaggctctgtacaccatggaggagaagctcgctctaaaaataaccctgtccctggtggatccactacgggtctatgctgcccatgtaaggaggcaaggcctggggacacccgagatgcctggttataattaaccccaacacctgctgcccccccccccccaacacctgctgcctgagcctgagcggttaccccaccccggtgcctgggtcttaggctctgtacaccatggaggagaagctcgctctaaaaataaccctgtccctggtggaccactacgggtctaggctgcccatgtaaggaggcaaggcctggggacacccgagatgcctggttataattaaccccaacacctgctgccccccccccccaacacctgctgcctgagcctgagcggttaccccaccccggtgcctgggtcttaggctctgtacaccatggaggagaagctcgctctaaaaataaccctgtccctggtcctccctggggacagcccctcctggctagtcacaccctgtaggctcctctatataacccaggggcacaggggctgcccccgggtcacctgcagaagttggtcgtgaggcactgggcaggtaagtatcaaggttacaagacaggtttaaggagaccaatagaaactgggcttgtcgagacagagaagactcttgcgtttctgataggcacctattggtcttactgacatccactttgcctttctctccacaggtgtccactcccagttcaattacagcgcgtggtaccaccatggcagcagcagccgccgcagccgccgagcagcagtcaagcaatggaccagtgaaaaaatcaatgagagaaaaagccgtcgagaggagatcagtgaataaggagcacaacagcaatttcaaagccggctacatccctattgacgaagatcgcctgcataagacaggcctgagggggcgcaaaggaaacctggcaatctgcgtcatcattctgctgtttatcctggccgtgattaatctgatcattactctggtgatttgggctgtcatccgcattggcccaaacgggtgtgactctatggagttccacgaaagtggcctgctgcgatttaagcaggtgtccgatatgggggtcatccatccactgtacaaatctactgtcggcgggcggagaaacgagaatctggtgatcaccgggaacaatcagcccattgtgttccagcagggaaccacaaagctgtctgtggaaaacaataaaacatcaatcactagcgacattggcatgcagttctttgatccccggacccagaatatcctgttcagtaccgactatgagacacacgaatttcatctgccttccggggtgaagtctctgaacgtccagaaagccagcactgagagaatcaccagtaacgctacatcagacctgaatatcaaggtggatggacgagctattgtccggggaaatgagggcgtgttcatcatgggcaagacaattgaatttcacatgggaggcaacatggagctgaaagcagaaaacagcatcattctgaatgggagcgtgatggtctccactaccagactgcccagctcctctagtggagaccagctggggtccggagattgggtcaggtataagctgtgcatgtgtgccgatggcaccctgtttaaagtgcaggtcaccagccagaatatgggatgtcagattagcgataacccttgtgggaatactcattaaaagcttggccgcaataaaagatctttattttcattagatctgtgtgttggttttttgtgtgtcctgcaggggcgcgcctctagagcatggctacgtagataagtagcatggcgggttaatcattaactacaaggaacccctagtgatggagttggccactccctctctgcgcgctcgctcgctcactgaggccgggcgaccaaaggtcgcccgacgcccgggctttgccc

SEQ ID NO: 6 - DNA, 714 bp, Artificial Sequence
  Primer
  misc_feature: tMCK promoter
ccactacgggtctaggctgcccatgtaaggaggcaaggcctggggacacccgagatgcctggttataattaaccccaacacctgctgcccccccccccccaacacctgctgcctgagcctgagcggttaccccaccccggtgcctgggtcttaggctctgtacaccatggaggagaagctcgctctaaaaataaccctgtccctggtggatccactacgggtctatgctgcccatgtaaggaggcaaggcctggggacacccgagatgcctggttataattaaccccaacacctgctgcccccccccccccaacacctgctgcctgagcctgagcggttaccccaccccggtgcctgggtcttaggctctgtacaccatggaggagaagctcgctctaaaaataaccctgtccctggtggaccactacgggtctaggctgcccatgtaaggaggcaaggcctggggacacccgagatgcctggttataattaaccccaacacctgctgccccccccccccaacacctgctgcctgagcctgagcggttaccccaccccggtgcctgggtcttaggctctgtacaccatggaggagaagctcgctctaaaaataaccctgtccctggtcctccctggggacagcccctcctggctagtcacaccctgtaggctcctctatataacccaggggcacaggggctgcccccgggtcac

SEQ ID NO: 7 - DNA, 296 bp, Artificial Sequence
  Primer
  misc_feature: miR29c
ggccggcctgtttgaatgaggcttcagtactttacagaatcgttgcctgcacatcttggaaacacttgctgggattacttcttcaggttaacccaacagaaggctcgagaaggtatattgctgttgacagtgagcgcaaccgatttcaaatggtgctagagtgaagccacagatgtctagcaccatttgaaatcggttatgcctactgcctcggaattcaaggggctactttaggagcaattatcttgtttactaaaactgaataccttgctatctctttgatacattggccggcc

SEQ ID NO: 8 - DNA, 3384 bp, Artificial Sequence
  Primer
  misc_feature: pAAV.CMV.Mir29C
cagcagctgcgcgctcgctcgctcactgaggccgcccgggcaaagcccgggcgtcgggcgacctttggtcgcccggcctcagtgagcgagcgagcgcgcagagagggagtggggttaaactcgttacataacttacggtaaatggcccgcctggctgaccgcccaacgacccccgcccattgacgtcaataatgacgtatgttcccatagtaacgccaatagggactttccattgacgtcaatgggtggagtatttacggtaaactgcccacttggcagtacatcaagtgtatcatatgccaagtacgccccctattgacgtcaatgacggtaaatggcccgcctggcattatgcccagtacatgaccttatgggactttcctacttggcagtacatctacgtattagtcatcgctattaccatggtgatgcggttttggcagtacatcaatgggcgtggatagcggtttgactcacggggatttccaagtctccaccccattgacgtcaatgggagtttgttttggcaccaaaatcaacgggactttccaaaatgtcgtaacaactccgccccattgacgcaaatgggcggtaggcgtgtacggtgggaggtctatataagcagagctcgtttagtgaaccgtcagatcgcctggagacgccatccacgctgttttgacctccatagaagacaccgggaccgatccagcctccggactctagaggatccggtactcgaggaactgaaaaaccagaaagttaactggtaagtttagtctttttgtcttttatttcaggtcccggatccggtggtggtgcaaatcaaagaactgctcctcagtggatgttgcctttacttctaggcctgtacggaagtgttacttctgctctaaaagctgcggaattgtacccggggccgatccaccggtctttttcgcaacgggtttgccgccagaacacaggtaagtgccgtgtgtggttcccgcgggcggcgacggggcccgtgcgtcccagcgcacatgttcggcgaggcggggcctgcgagcgcggccaccgagaatcggacgggggtagtctcaagctggccggcctgtttgaatgaggcttcagtactttacagaatcgttgcctgcacatcttggaaacacttgctgggattacttcttcaggttaacccaacagaaggctcgagaaggtatattgctgttgacagtgagcgcaaccgatttcaaatggtgctagagtgaagccacagatgtctagcaccatttgaaatcggttatgcctactgcctcggaattcaaggggctactttaggagcaattatcttgtttactaaaactgaataccttgctatctctttgatacattggccggcctgctctggtgcctggcctcgcgccgccgtgtatcgccccgccctgggcggcaaggctggcccggtcggcaccagttgcgtgagcggaaagatggccgcttcccggccctgctgcagggagctcaaaatggaggacgcggcgctcgggagagcgggcgggtgagtcacccacacaaaggaaaagggcctttccgtcctcagccgtcgcttcatgtgactccacggagtaccgggcgccgtccaggcacctcgattagttctcgagcttttggagtacgtcgtctttaggttggggggaggggttttatgcgatggagtttccccacactgagtgggtggagactgaagttaggccagcttggcacttgatgtaattctccttggaatttgccctttttgagtttggatcttggttcattctcaagcctcagacagtggttcaaagtttttttcttccatttcaggtgtcgtgaaaagctagcgctaccggactcagatctcgagctcaagctgcggggatccagacatgataagatacattgatgagtttggacaaaccacaactagaatgcagtgaaaaaaatgctttatttgtgaaatttgtgatgctattgctttatttgtaaccattataagctgcaataaacaagttaacaacaacaattgcattcattttatgtttcaggttcagggggaggtgtgggaggttttttcactagtagcatggctacgtagataagtagcatggcgggttaatcattaactacaaggaacccctagtgatggagttggccactccctctctgcgcgctcgctcgctcactgaggccgggcgaccaaaggtcgcccgacgcccgggctttgcccgggcggcctcagtgagcgagcgagcgcgccagctggcgtaatagcgaagaggcccgcaccgatcgcccttcccaacagttgcgcagcctgaatggcgaatggaattccagacgattgagcgtcaaaatgtaggtatttccatgagcgtttttcctgttgcaatggctggcggtaatattgttctggatattaccagcaaggccgatagtttgagttcttctactcaggcaagtgatgttattactaatcaaagaagtattgcgacaacggttaatttgcgtgatggacagactcttttactcggtggcctcactgattataaaaacacttctcaggattctggcgtaccgttcctgtctaaaatccctttaatcggcctcctgtttagctcccgctctgattctaacgaggaaagcacgttatacgtgctcgtcaaagcaaccatagtacgcgccctgtagcggcgcattaagcgcggcgggtgtggtggttacgcgcagcgtgaccgctacacttgccagcgccctagcgcccgctcctttcgctttcttcccttcctttctcgccacgttcgccggctttccccgtcaagctctaaatcgggggctccctttagggttccgatttagtgctttacggcacctcgaccccaaaaaacttgattagggtgatggttcacgtagtgggccatcgccctgatagacggtttttcgccctttgacgttggagtccacgttctttaatagtggactcttgttccaaactggaacaacactcaaccctatctcggtctattcttttgatttataagggattttgccgatttcggcctattggttaaaaaatgagctgatttaacaaaaatttaacgcgaattttaacaaaatattaacgtttacaatttaaatatttgcttatacaatcttcctgtttttggggcttttctgattatcaaccggggtacatatgattgacatgctagttttacgattaccgttcatcgattctcttgtttgctccagactctcaggcaatgacctgatagcctttgtagagacctctcaaaaatagctaccctctccggcatgaatttatcagctagaacggttgaatatcatattgatggtgatttgactgtc

SEQ ID NO: 9 - DNA, 296 bp, Artificial Sequence; identical to SEQ ID NO: 7
  Primer
  misc_feature: miR29c

SEQ ID NO: 10 - DNA, 23 bp, Artificial Sequence
  Primer
  misc_feature: tMCK forward primer
acccgagatgcctggttataatt

SEQ ID NO: 11 - DNA, 24 bp, Artificial Sequence
  Primer
  misc_feature: tMCK reverse primer
tccatggtgtacagagcctaagac

SEQ ID NO: 12 - DNA, 25 bp, Artificial Sequence
  Primer
  misc_feature: tMCK probe
  misc_feature (1)..(1): 5' FAM
  misc_feature (25)..(25): 3' TAMRA
ctgctgcctgagcctgagcggttac

SEQ ID NO: 13 - DNA, 20 bp, Artificial Sequence
  Primer
  misc_feature: tMCK intron Forward Primer
gtgaggcactgggcaggtaa

SEQ ID NO: 14 - DNA, 22 bp, Artificial Sequence
  Primer
  misc_feature: tMCK intron Reverse Primer
acctgtggagagaaaggcaaag

SEQ ID NO: 15 - DNA, 39 bp, Artificial Sequence
  Primer
  misc_feature: tMCK intron Probe
  misc_feature (1)..(1): 5' 6FAM
  misc_feature (39)..(39): 3' TAMRA
atcaaggttacaagacaggtttaaggagaccaatagaaa

SEQ ID NO: 16 - DNA, 21 bp, Artificial Sequence
  Primer
ccaacacctgctgcctctaaa

SEQ ID NO: 17 - DNA, 19 bp, Artificial Sequence
  Primer
  misc_feature: MHCK7 reverse primer
gtcccccacagccttgttc

SEQ ID NO: 18 - DNA, 23 bp, Artificial Sequence
  Primer
  misc_feature: MHCK7 probe
  misc_feature (1)..(1): 5' FAM
  misc_feature (9)..(9): Zen
  misc_feature (23)..(23): 3IABKFQ
tggatcccctgcatgcgaagatc